European Patent Specification EP 3 926 043 B1, published February 19, 2025. Title: SPECIAL ENZYME FOR GALACTOOLIGOSACCHARIDE PRODUCTION AS WELL AS PREPARATION AND APPLICATION THEREOF. Applicant: Tianjin University of Science and Technology. The sequence listing filed with the application follows.

SEQUENCE LISTING (71 sequences)

SEQ ID NO: 1 - DNA, 5133 bp, B. circulans B2301
atgaaaagcacgacgagcgccgccggcaaaagcgtcagctataacgacggcgaacgccgcgtcaactttgaaaactggcgctttcagcgcgaaacgaacggcagcatcgccggcgcccagaacccgggctttgacgacagcagctggcgcaaactgaacctgccgcatgaatggagcatcgacctggactttaacaaaaacagcctggccacgcatgaaggcggctatctggacggcggcatcggctggaaccgcaaaacgtttacgatcccggaaagcatgaaaggcaaacgctttagcctggacatcgacggcgtctatatgtatagcacgacgtatctgaacgcctttgtcctgggcacgtatccgtttggctataacggcgaaagctatgacatcagcgacaaactgtataaagacggccgcgccaacgtcctggtcgtcaaagtcaacacgaaccagccgagcggccgctggtatagcggcagcagcatctatcgcaacgtctatctgacggtcacggacccgatccatgtcgcccgctatggcacgtttgtcacgacgccgaacctggaaaaaagcatcaaagaagaccgcgacgccgtcaacatcaaaacgaaaatcagcaacgccgaagccaaacaggtcaaaatcgccgacaaaagcacgatctatgacggcgccggcaacacggtccagacggtcgaaacggaagaaaaaacggccgccggcgccacggtcacgccgtttgaacagaacacggtcatcaaacagccgaaactgtggagcatcgacaaaccgtatcgctataacctggtcacggaagtcatcgtcggcggccagacggtcgacacgtatgaaacgaaatttggcgtccgctattttaaatttgacgaaaacgaaggctatagcctgaacggcgaatttatgaaactgcatggcgtcagcatgcatcatgacctggccggcggcgccgccctgacgaacgcccgcggcgtcgaacgccagatgcagatcatgaaagacgtcggcgtcaacgccatccgcgtcacgcataacccggccagcccggaactgggcctggaatttgccgccaacaaactgctgatcatcgaagaagcctttgacagctgggcccagagcaaaaaaccgtatgactatggccgcttttttaacgcctgggccgaacatgacatcaaagaaatggtcgaccgcggcaaaaacgaaccggccatcatcatgtggagcatcggcaacgaaatctatgacacgacgaacgccgccggcgtcgaaacggcccgcaacctggtcggctgggtcaaagaaatcgacacgacgccgcgcgccacgatcggcgaagacaaaacgcgcggcgacaacgtcacgccgatcaacagctatatcaaagaaatctttaacatcgtcgacgtcgtcggcctgaactatagcgaaaacaactatgacggctatcataaacagaacccgagctggaaactgtatggcagcgaaacgagcagcgccacgcgcagccgcggcgtctatacgcagccgtatcagtataaccatgacacgaaatatgccgacctgcagcagagcagctatgacaacgactatgtcggctggggccgcacggcccaggacgcctggaaatatgaccgcgacctgaaacatatcgccggccagtttatctggacgggctttgactatatcggcgaaccgacgccgtattataacagctatccggccaaaagcagctattttggcgccgtcgacacggccggctttccgaaagacatcttttattattatcagagccagtggaaaaaagaaccgatggtccatctgctgccgcattggaactggaaagaaggcgaaaaagtccgcgtcctggcctatacgaacgccagcaaagtcgaactggtcctgaacggcgaaagcctgggcaacgaaaaatatgacaacaaacagacgagctggggcgccccgtataaagaaacgaaagacggcaaaacgtatctggaatgggccgtcaaaccgctgaaaccgggcaaatttgacgaagccgtcgccgaaaacggcaaagtcatcgcccgcgaccaggtcgtcacggccggcgaaccggccagcgtccgcctgacggccgaccgcaaagtcgtcaaagccgacggcacggaccatagctttatcacggccgacatcgtcgacagcaaaggcatcgtcgtcccggacgccgaccatctgatcacgtttaacgtcacgggccagggcgaactggccggcgtcgacaacggcaacgccagcagcgtcgaacgctataaagacaacaaacgcaaagcctttagcggcaaagccctggccatcgtccagagcagcaaactgagcggcaaaatcacggtccatgccagcgtcgccggcctgagcagcgacagcacgagcgtctttacggtcacgccggccgaccatgacaaaaaaatcgtcgccggcatcgacgacgtcaacctgacggtcgacgtcaacgaagccccgaaactgccgagcgaaatcaaagtctattatagcgacgaaagcgccgccgccaaaaacgtcacgtgggacgaagtcgacccgaaacagtatagcacggtcggcgaatttacggtcgaaggcagcgtcgaaggcacgagcctgaaagccaaagcctttgtcatcgtcaaaggcatcgtcgccgtcaaaccgtatagcacggccacgaaagtcggcgtccagccggtcctgccggaaaaagccacgctgctgtatagcgacggcacgacgaaaggcgccacggtcacgtgggacgaactgccggaagacaaactggccaaagaaggccgctttacggtcgaaggcagcgtcgaaggcacggacctgaaagccaacgtctatgtccgcgtcacgaacgaagtcaaaagcgtcaacatcatgctgcaggaacagggcagcgcctatccgaaactggaagccacgtttacgaacccggccgacaacctgcagcatctgaacgacggcatcaaaagctatacgaacaaccaggtcaaccgctggacgaactggacgcgcacgccgcgcgacgccggcgacagcatcacggtcaactttggcaaaaaacatgtcatcaacaacctggacctgtttgtctttacggacagcggcacggtcgtcccggaaaaagccgaagtccagtattgggacggcacggccgtcaaagacgtcgaaaacctgacgcagccgagcccgtatgtcgtcgaaaaaaacgaactgacgtttgacgccgtcgccacggaaaaactgaaatttcatctgacgccgagcgtcaaaggcaaatttctggccctgacggaagccgaagtctatgccgaccagatcgtcgacggcgaaacggccaaactgcagagcatcacggtcaacggcaaagccctggaaggctttgaccatgccaaaaaaaactatgaactggtcctgccgtatggcagcgaactgccgaaaatcgaagccgccgccgccgacaacgccacggtcacgatcctgccggcctttagctatccgggcacggccaaactgtttgtcacgagcgaagacggcaaagtcacgacggaatatagcatcggcgtcagcacggaagaaccgaaactggtcagcgccgaactgagcgccgacaaaacgaacgtcatggaagacgacatcatcgacctgaaagtcatcggcctgtttgaaagcaaagaaaaaatcgacgtcacggacagccagccgacgtatgaatttgaccagcagatcatcaaaatcgaaggcaacaaactgtatgccctggaaacgggcaacgtcaaagtcaaagtcacggtcacgtataaaggcgtcagcgtcacgacgccggccctggaatttacgatcgccaaacatccggccccgaaatatatcacgagcctggaaccggtcacggtcgtcgtcaaaaaaggcgaagccccggaactgccggccacggtcgtcgcccattataaccgcggcatcccgcgcgacgtcaaagtcaaatgggaacgcatccatccgagcaaatatcagcagctgggcgaatttacggtcagcggcatggtcgaaggcacggacatcaaagcccaggccaaagtcgccgtcaaaggcgccgtcatcgtcgaagacatccgcatggccgtcctgctgaaacagatgccgcagctgccgggcaaagtcacggtctattatagcgacggcgccgaagaacagcgcgccgtcaaatgggaagaaatcccgcaggaagaactggaaaaagtcggcgaatttaaagtcaacggcgacgtcaacggcgtcaaactgaaagccacggccacgatccgcgtcacggacgaagtcggcgccgaacagaacatcagccgcgccaaaaacggctatgaatatccgaaagccgaagccagctttacgaacgacggcccgggcagcagcgaccgcatcgaagccatcaacgacgacgtcatcagctatgaagccaacccgcataaccgctggacgaactggcagccggccccgcgcgtcggcgacctggtctttacgacgtttggcgactatgaaccgacggaatatgacgtcgacagcatggaaatccattggtttgccgaccatggcacgagctatccggaacgctttcagatcgaatataaaagcggcgacagctggaaagaagtcacgagcctgaaaagcgacccggccagcccggccctgggcaaagccaacgtctatagctttgaccgcgtcaaaacgagcgccatccgcgtcaaaatgacggcccaggccggcaaaagcctggccatcacggaactgaaagtctttagcaaatggccgaaagccggcacggaaccggacgtcacggacatcaaagtcggcggcaaaagcatcctggaagaatttgaacaggaaggcgaccattatgaagccacgatcgacgtcggcgacgccaacgtcatgccgaaaatctatgtcaaagccaaagaccagacgagcatcagcatcgtcccggccgtcacgagcgtcagcacggccaaagtcatcgccgaagacggcgacggcaaaaaagtcaaagtctatagcatccataaaagctataaataa

SEQ ID NO: 2 - protein, 1710 aa, B. circulans B2301
MKSTTSAAGKSVSYNDGERRVNFENWRFQRETNGSIAGAQNPGFDDSSWRKLNLPHEWSIDLDFNKNSLATHEGGYLDGGIGWNRKTFTIPESMKGKRFSLDIDGVYMYSTTYLNAFVLGTYPFGYNGESYDISDKLYKDGRANVLVVKVNTNQPSGRWYSGSSIYRNVYLTVTDPIHVARYGTFVTTPNLEKSIKEDRDAVNIKTKISNAEAKQVKIADKSTIYDGAGNTVQTVETEEKTAAGATVTPFEQNTVIKQPKLWSIDKPYRYNLVTEVIVGGQTVDTYETKFGVRYFKFDENEGYSLNGEFMKLHGVSMHHDLAGGAALTNARGVERQMQIMKDVGVNAIRVTHNPASPELGLEFAANKLLIIEEAFDSWAQSKKPYDYGRFFNAWAEHDIKEMVDRGKNEPAIIMWSIGNEIYDTTNAAGVETARNLVGWVKEIDTTPRATIGEDKTRGDNVTPINSYIKEIFNIVDVVGLNYSENNYDGYHKQNPSWKLYGSETSSATRSRGVYTQPYQYNHDTKYADLQQSSYDNDYVGWGRTAQDAWKYDRDLKHIAGQFIWTGFDYIGEPTPYYNSYPAKSSYFGAVDTAGFPKDIFYYYQSQWKKEPMVHLLPHWNWKEGEKVRVLAYTNASKVELVLNGESLGNEKYDNKQTSWGAPYKETKDGKTYLEWAVKPLKPGKFDEAVAENGKVIARDQVVTAGEPASVRLTADRKVVKADGTDHSFITADIVDSKGIVVPDADHLITFNVTGQGELAGVDNGNASSVERYKDNKRKAFSGKALAIVQSSKLSGKITVHASVAGLSSDSTSVFTVTPADHDKKIVAGIDDVNLTVDVNEAPKLPSEIKVYYSDESAAAKNVTWDEVDPKQYSTVGEFTVEGSVEGTSLKAKAFVIVKGIVAVKPYSTATKVGVQPVLPEKATLLYSDGTTKGATVTWDELPEDKLAKEGRFTVEGSVEGTDLKANVYVRVTNEVKSVNIMLQEQGSAYPKLEATFTNPADNLQHLNDGIKSYTNNQVNRWTNWTRTPRDAGDSITVNFGKKHVINNLDLFVFTDSGTVVPEKAEVQYWDGTAVKDVENLTQPSPYVVEKNELTFDAVATEKLKFHLTPSVKGKFLALTEAEVYADQIVDGETAKLQSITVNGKALEGFDHAKKNYELVLPYGSELPKIEAAAADNATVTILPAFSYPGTAKLFVTSEDGKVTTEYSIGVSTEEPKLVSAELSADKTNVMEDDIIDLKVIGLFESKEKIDVTDSQPTYEFDQQIIKIEGNKLYALETGNVKVKVTVTYKGVSVTTPALEFTIAKHPAPKYITSLEPVTVVVKKGEAPELPATVVAHYNRGIPRDVKVKWERIHPSKYQQLGEFTVSGMVEGTDIKAQAKVAVKGAVIVEDIRMAVLLKQMPQLPGKVTVYYSDGAEEQRAVKWEEIPQEELEKVGEFKVNGDVNGVKLKATATIRVTDEVGAEQNISRAKNGYEYPKAEASFTNDGPGSSDRIEAINDDVISYEANPHNRWTNWQPAPRVGDLVFTTFGDYEPTEYDVDSMEIHWFADHGTSYPERFQIEYKSGDSWKEVTSLKSDPASPALGKANVYSFDRVKTSAIRVKMTAQAGKSLAITELKVFSKWPKAGTEPDVTDIKVGGKSILEEFEQEGDHYEATIDVGDANVMPKIYVKAKDQTSISIVPAVTSVSTAKVIAEDGDGKKVKVYSIHKSYK

SEQ ID NO: 3 - DNA, 3672 bp, Artificial sequence
  The sequence is synthesized
atgaaaagcacgacgagcgccgccggcaaaagcgtcagctataacgacggcgaacgccgcgtcaactttgaaaactggcgctttcagcgcgaaacgaacggcagcatcgccggcgcccagaacccgggctttgacgacagcagctggcgcaaactgaacctgccgcatgaatggagcatcgacctggactttaacaaaaacagcctggccacgcatgaaggcggctatctggacggcggcatcggctggaaccgcaaaacgtttacgatcccggaaagcatgaaaggcaaacgctttagcctggacatcgacggcgtctatatgtatagcacgacgtatctgaacgcctttgtcctgggcacgtatccgtttggctataacggcgaaagctatgacatcagcgacaaactgtataaagacggccgcgccaacgtcctggtcgtcaaagtcaacacgaaccagccgagcggccgctggtatagcggcagcagcatctatcgcaacgtctatctgacggtcacggacccgatccatgtcgcccgctatggcacgtttgtcacgacgccgaacctggaaaaaagcatcaaagaagaccgcgacgccgtcaacatcaaaacgaaaatcagcaacgccgaagccaaacaggtcaaaatcgccgacaaaagcacgatctatgacggcgccggcaacacggtccagacggtcgaaacggaagaaaaaacggccgccggcgccacggtcacgccgtttgaacagaacacggtcatcaaacagccgaaactgtggagcatcgacaaaccgtatcgctataacctggtcacggaagtcatcgtcggcggccagacggtcgacacgtatgaaacgaaatttggcgtccgctattttaaatttgacgaaaacgaaggctatagcctgaacggcgaatttatgaaactgcatggcgtcagcatgcatcatgacctggccggcggcgccgccctgacgaacgcccgcggcgtcgaacgccagatgcagatcatgaaagacgtcggcgtcaacgccatccgcgtcacgcataacccggccagcccggaactgggcctggaatttgccgccaacaaactgctgatcatcgaagaagcctttgacagctgggcccagagcaaaaaaccgtatgactatggccgcttttttaacgcctgggccgaacatgacatcaaagaaatggtcgaccgcggcaaaaacgaaccggccatcatcatgtggagcatcggcaacgaaatctatgacacgacgaacgccgccggcgtcgaaacggcccgcaacctggtcggctgggtcaaagaaatcgacacgacgccgcgcgccacgatcggcgaagacaaaacgcgcggcgacaacgtcacgccgatcaacagctatatcaaagaaatctttaacatcgtcgacgtcgtcggcctgaactatagcgaaaacaactatgacggctatcataaacagaacccgagctggaaactgtatggcagcgaaacgagcagcgccacgcgcagccgcggcgtctatacgcagccgtatcagtataaccatgacacgaaatatgccgacctgcagcagagcagctatgacaacgactatgtcggctggggccgcacggcccaggacgcctggaaatatgaccgcgacctgaaacatatcgccggccagtttatctggacgggctttgactatatcggcgaaccgacgccgtattataacagctatccggccaaaagcagctattttggcgccgtcgacacggccggctttccgaaagacatcttttattattatcagagccagtggaaaaaagaaccgatggtccatctgctgccgcattggaactggaaagaaggcgaaaaagtccgcgtcctggcctatacgaacgccagcaaagtcgaactggtcctgaacggcgaaagcctgggcaacgaaaaatatgacaacaaacagacgagctggggcgccccgtataaagaaacgaaagacggcaaaacgtatctggaatgggccgtcaaaccgctgaaaccgggcaaatttgacgaagccgtcgccgaaaacggcaaagtcatcgcccgcgaccaggtcgtcacggccggcgaaccggccagcgtccgcctgacggccgaccgcaaagtcgtcaaagccgacggcacggaccatagctttatcacggccgacatcgtcgacagcaaaggcatcgtcgtcccggacgccgaccatctgatcacgtttaacgtcacgggccagggcgaactggccggcgtcgacaacggcaacgccagcagcgtcgaacgctataaagacaacaaacgcaaagcctttagcggcaaagccctggccatcgtccagagcagcaaactgagcggcaaaatcacggtccatgccagcgtcgccggcctgagcagcgacagcacgagcgtctttacggtcacgccggccgaccatgacaaaaaaatcgtcgccggcatcgacgacgtcaacctgacggtcgacgtcaacgaagccccgaaactgccgagcgaaatcaaagtctattatagcgacgaaagcgccgccgccaaaaacgtcacgtgggacgaagtcgacccgaaacagtatagcacggtcggcgaatttacggtcgaaggcagcgtcgaaggcacgagcctgaaagccaaagcctttgtcatcgtcaaaggcatcgtcgccgtcaaaccgtatagcacggccacgaaagtcggcgtccagccggtcctgccggaaaaagccacgctgctgtatagcgacggcacgacgaaaggcgccacggtcacgtgggacgaactgccggaagacaaactggccaaagaaggccgctttacggtcgaaggcagcgtcgaaggcacggacctgaaagccaacgtctatgtccgcgtcacgaacgaagtcaaaagcgtcaacatcatgctgcaggaacagggcagcgcctatccgaaactggaagccacgtttacgaacccggccgacaacctgcagcatctgaacgacggcatcaaaagctatacgaacaaccaggtcaaccgctggacgaactggacgcgcacgccgcgcgacgccggcgacagcatcacggtcaactttggcaaaaaacatgtcatcaacaacctggacctgtttgtctttacggacagcggcacggtcgtcccggaaaaagccgaagtccagtattgggacggcacggccgtcaaagacgtcgaaaacctgacgcagccgagcccgtatgtcgtcgaaaaaaacgaactgacgtttgacgccgtcgccacggaaaaactgaaatttcatctgacgccgagcgtcaaaggcaaatttctggccctgacggaagccgaagtctatgccgaccagatcgtcgacggcgaaacggccaaactgcagagcatcacggtcaacggcaaagccctggaaggctttgaccatgccaaaaaaaactatgaactggtcctgccgtatggcagcgaactgccgaaaatcgaagccgccgccgccgacaacgccacggtcacgatcctgccggcctttagctatccgggcacggccaaactgtttgtcacgagcgaagacggcaaagtcacgacggaatatagcatcggcgtcagcacggaagaaccgaaactggtcagcgccgaactgagctaa

SEQ ID NO: 4 - protein, 1223 aa, Artificial sequence
  The sequence is synthesized
MKSTTSAAGKSVSYNDGERRVNFENWRFQRETNGSIAGAQNPGFDDSSWRKLNLPHEWSIDLDFNKNSLATHEGGYLDGGIGWNRKTFTIPESMKGKRFSLDIDGVYMYSTTYLNAFVLGTYPFGYNGESYDISDKLYKDGRANVLVVKVNTNQPSGRWYSGSSIYRNVYLTVTDPIHVARYGTFVTTPNLEKSIKEDRDAVNIKTKISNAEAKQVKIADKSTIYDGAGNTVQTVETEEKTAAGATVTPFEQNTVIKQPKLWSIDKPYRYNLVTEVIVGGQTVDTYETKFGVRYFKFDENEGYSLNGEFMKLHGVSMHHDLAGGAALTNARGVERQMQIMKDVGVNAIRVTHNPASPELGLEFAANKLLIIEEAFDSWAQSKKPYDYGRFFNAWAEHDIKEMVDRGKNEPAIIMWSIGNEIYDTTNAAGVETARNLVGWVKEIDTTPRATIGEDKTRGDNVTPINSYIKEIFNIVDVVGLNYSENNYDGYHKQNPSWKLYGSETSSATRSRGVYTQPYQYNHDTKYADLQQSSYDNDYVGWGRTAQDAWKYDRDLKHIAGQFIWTGFDYIGEPTPYYNSYPAKSSYFGAVDTAGFPKDIFYYYQSQWKKEPMVHLLPHWNWKEGEKVRVLAYTNASKVELVLNGESLGNEKYDNKQTSWGAPYKETKDGKTYLEWAVKPLKPGKFDEAVAENGKVIARDQVVTAGEPASVRLTADRKVVKADGTDHSFITADIVDSKGIVVPDADHLITFNVTGQGELAGVDNGNASSVERYKDNKRKAFSGKALAIVQSSKLSGKITVHASVAGLSSDSTSVFTVTPADHDKKIVAGIDDVNLTVDVNEAPKLPSEIKVYYSDESAAAKNVTWDEVDPKQYSTVGEFTVEGSVEGTSLKAKAFVIVKGIVAVKPYSTATKVGVQPVLPEKATLLYSDGTTKGATVTWDELPEDKLAKEGRFTVEGSVEGTDLKANVYVRVTNEVKSVNIMLQEQGSAYPKLEATFTNPADNLQHLNDGIKSYTNNQVNRWTNWTRTPRDAGDSITVNFGKKHVINNLDLFVFTDSGTVVPEKAEVQYWDGTAVKDVENLTQPSPYVVEKNELTFDAVATEKLKFHLTPSVKGKFLALTEAEVYADQIVDGETAKLQSITVNGKALEGFDHAKKNYELVLPYGSELPKIEAAAADNATVTILPAFSYPGTAKLFVTSEDGKVTTEYSIGVSTEEPKLVSAELS

SEQ ID NO: 5 - DNA, 2436 bp, Artificial Sequence
  The sequence is synthesized
atgaaaagcacgacgagcgccgccggcaaaagcgtcagctataacgacggcgaacgccgcgtcaactttgaaaactggcgctttcagcgcgaaacgaacggcagcatcgccggcgcccagaacccgggctttgacgacagcagctggcgcaaactgaacctgccgcatgaatggagcatcgacctggactttaacaaaaacagcctggccacgcatgaaggcggctatctggacggcggcatcggctggaaccgcaaaacgtttacgatcccggaaagcatgaaaggcaaacgctttagcctggacatcgacggcgtctatatgtatagcacgacgtatctgaacgcctttgtcctgggcacgtatccgtttggctataacggcgaaagctatgacatcagcgacaaactgtataaagacggccgcgccaacgtcctggtcgtcaaagtcaacacgaaccagccgagcggccgctggtatagcggcagcagcatctatcgcaacgtctatctgacggtcacggacccgatccatgtcgcccgctatggcacgtttgtcacgacgccgaacctggaaaaaagcatcaaagaagaccgcgacgccgtcaacatcaaaacgaaaatcagcaacgccgaagccaaacaggtcaaaatcgccgacaaaagcacgatctatgacggcgccggcaacacggtccagacggtcgaaacggaagaaaaaacggccgccggcgccacggtcacgccgtttgaacagaacacggtcatcaaacagccgaaactgtggagcatcgacaaaccgtatcgctataacctggtcacggaagtcatcgtcggcggccagacggtcgacacgtatgaaacgaaatttggcgtccgctattttaaatttgacgaaaacgaaggctatagcctgaacggcgaatttatgaaactgcatggcgtcagcatgcatcatgacctggccggcggcgccgccctgacgaacgcccgcggcgtcgaacgccagatgcagatcatgaaagacgtcggcgtcaacgccatccgcgtcacgcataacccggccagcccggaactgggcctggaatttgccgccaacaaactgctgatcatcgaagaagcctttgacagctgggcccagagcaaaaaaccgtatgactatggccgcttttttaacgcctgggccgaacatgacatcaaagaaatggtcgaccgcggcaaaaacgaaccggccatcatcatgtggagcatcggcaacgaaatctatgacacgacgaacgccgccggcgtcgaaacggcccgcaacctggtcggctgggtcaaagaaatcgacacgacgccgcgcgccacgatcggcgaagacaaaacgcgcggcgacaacgtcacgccgatcaacagctatatcaaagaaatctttaacatcgtcgacgtcgtcggcctgaactatagcgaaaacaactatgacggctatcataaacagaacccgagctggaaactgtatggcagcgaaacgagcagcgccacgcgcagccgcggcgtctatacgcagccgtatcagtataaccatgacacgaaatatgccgacctgcagcagagcagctatgacaacgactatgtcggctggggccgcacggcccaggacgcctggaaatatgaccgcgacctgaaacatatcgccggccagtttatctggacgggctttgactatatcggcgaaccgacgccgtattataacagctatccggccaaaagcagctattttggcgccgtcgacacggccggctttccgaaagacatcttttattattatcagagccagtggaaaaaagaaccgatggtccatctgctgccgcattggaactggaaagaaggcgaaaaagtccgcgtcctggcctatacgaacgccagcaaagtcgaactggtcctgaacggcgaaagcctgggcaacgaaaaatatgacaacaaacagacgagctggggcgccccgtataaagaaacgaaagacggcaaaacgtatctggaatgggccgtcaaaccgctgaaaccgggcaaatttgacgaagccgtcgccgaaaacggcaaagtcatcgcccgcgaccaggtcgtcacggccggcgaaccggccagcgtccgcctgacggccgaccgcaaagtcgtcaaagccgacggcacggaccatagctttatcacggccgacatcgtcgacagcaaaggcatcgtcgtcccggacgccgaccatctgatcacgtttaacgtcacgggccagggcgaactggccggcgtcgacaacggcaacgccagcagcgtcgaacgctataaagacaacaaacgcaaagcctttagcggcaaagccctggccatcgtccagagcagcaaactgagcggcaaaatcacggtccatgccagcgtcgccggcctgagcagcgacagcacgtaa

SEQ ID NO: 6 - protein, 811 aa, Artificial Sequence
  The sequence is synthesized
MKSTTSAAGKSVSYNDGERRVNFENWRFQRETNGSIAGAQNPGFDDSSWRKLNLPHEWSIDLDFNKNSLATHEGGYLDGGIGWNRKTFTIPESMKGKRFSLDIDGVYMYSTTYLNAFVLGTYPFGYNGESYDISDKLYKDGRANVLVVKVNTNQPSGRWYSGSSIYRNVYLTVTDPIHVARYGTFVTTPNLEKSIKEDRDAVNIKTKISNAEAKQVKIADKSTIYDGAGNTVQTVETEEKTAAGATVTPFEQNTVIKQPKLWSIDKPYRYNLVTEVIVGGQTVDTYETKFGVRYFKFDENEGYSLNGEFMKLHGVSMHHDLAGGAALTNARGVERQMQIMKDVGVNAIRVTHNPASPELGLEFAANKLLIIEEAFDSWAQSKKPYDYGRFFNAWAEHDIKEMVDRGKNEPAIIMWSIGNEIYDTTNAAGVETARNLVGWVKEIDTTPRATIGEDKTRGDNVTPINSYIKEIFNIVDVVGLNYSENNYDGYHKQNPSWKLYGSETSSATRSRGVYTQPYQYNHDTKYADLQQSSYDNDYVGWGRTAQDAWKYDRDLKHIAGQFIWTGFDYIGEPTPYYNSYPAKSSYFGAVDTAGFPKDIFYYYQSQWKKEPMVHLLPHWNWKEGEKVRVLAYTNASKVELVLNGESLGNEKYDNKQTSWGAPYKETKDGKTYLEWAVKPLKPGKFDEAVAENGKVIARDQVVTAGEPASVRLTADRKVVKADGTDHSFITADIVDSKGIVVPDADHLITFNVTGQGELAGVDNGNASSVERYKDNKRKAFSGKALAIVQSSKLSGKITVHASVAGLSSDST

SEQ ID NO: 7 - DNA, 5133 bp, B. circulans ATCC 31382
atgagcaaaacgacgagcgccgccggcaacagcgtcagctatgacggcgaacgccgcgtcaactttaacgaaaactggcgctttcagcgcgaaacgaacggcagcatcgccggcgcccagaacccaggctttgacgacagcagctggcgcaaactgaacctgccgcatgactggagcatcgaactggactttaacaaaaacagcctggccacgcatgaaggcggctatctggacggcggcatcggctggtatcgcaaaacgtttacgatcccggaaagcatgaaaggcaaacgcatcagcctggactttgacggcgtctatatgaacagcacgacgtatctgaacggcgaagtcctgggcacgtatccgtttggctataacgcctttagctatgacatcagcgacaaactgtataaagacggccgcgccaacgtcctggtcgtcaaagtcaacaacacgcagccgagcagccgctggtatagcggcagcggcatctatcgcaacgtctatctgacggtcacggacccgatccatgtcgcccgctatggcacgtttgtcacgacgccgaacctggaaaaaagcatcaaagaagaccgcgccgacgtcaacatcaaaacgaaaatcagcaacgacgccgccgaagccaaacaggtcaaaatcaaaagcacgatctatgacggcgccggcaacacggtccagacggtcgaaacggaagaaaaaacggccgccgccggcacggtcacgccgtttgaacagaacacggtcatcaaacagccgaaactgtggagcatcgacaaaccgtatcgctataacctggtcacggaagtcatcgtcggcggccagacggtcgacacgtatgaaacgaaatttggcgtccgctattttaaatttgacgaaaacgaaggctttagcctgaacggcgaatatatgaaactgcatggcgtcagcatgcatcatgacctgggcgccctgggcgccgccacgaacgcccgcggcgtcgaacgccagatgcagatcatgaaagacatgggcgtcaacgccatccgcgtcacgcataacccggccagcccggaactgctggaagccgccaacaaactgggcctgtttatcatcgaagaagcctttgacagctgggcccagagcaaaaaaccgtatgactatggccgcttttttaacgcctgggccgaacatgacatcaaagaaatggtcgaccgcggcaaaaacgaaccggccatcatcatgtggagcatcggcaacgaaatctatgacacgacgaacgccgccggcgtcgaaacggcccgcaacctggtcggctgggtcaaagaaatcgacacgacgcgcccgacgacgatcggcgaagacaaaacgcgcggcgacaaagtcaacgtcacgccgatcaacagctatatcaaagaaatctttaacatcgtcgacgtcgtcggcctgaactatagcgaaaacaactatgacggctatcataaacagaacccgagctggaaactgtatggcagcgaaacgagcagcgccacgcgcagccgcggcgtctatacgcatccgtatcagtataaccagagcacgaaatatgccgacctgcagcagagcagctatgacaacgactatgtcggctggggccgcacggccgaagacgcctggaaatatgaccgcgacctgaaacatatcgccggccagtttatctggacgggctttgactatatcggcgaaccgacgccgtattataacagctatccggccaaaagcagctattttggcgccgtcgacacggccggctttccgaaagacatcttttattattatcagagccagtggaaaaaagaaccgatggtccatctgctgccgcattggaactggaaagaaggcgaaaaagtccgcgtcctggcctatacgaacgccagcaaagtcgaactggtcctgaacggcgaaagcctgggcgaaaaaaactatgacaacaaacagacgagctggggcgccccgtataaagaaacgaaagacggcaaaacgtatctggaatgggccgtcccgtttaaaccgggcaaactggaagccgtcgccaaagacgaaaacggcaaagtcatcgcccgcgaccaggtcgtcacggccggcgaaccggccagcgtccgcctgacggccgaccgcaaagtcgtcaaagccgacggcacggacctgagctttatcacggccgacatcgtcgacagcaaaggcatcgtcgtcccggacgccgaccatctgatcacgtttaacgtcacgggccagggcgaactggccggcgtcgacaacggcaacgccagcagcgtcgaacgctataaagacaacaaacgcaaagcctttagcggcaaagccctggccatcgtccagagcagcaaactgagcggcaaaatcacggtccatgccagcgtcgccggcctgagcagcgacagcacgagcgtctttacggtcacgccggccgaccatgacaaaaaaatcgtcgccggcatcgacgacgtcaacctgacggtcgacgtcaacgaagccccgaaactgccgagcgaaatcaaagtctattatagcgacgaaagcgccgccgccaaaaacgtcacgtgggacgaagtcgacccgaaacagtatagcacggtcggcgaatttacggtcgaaggcagcgtcgaaggcacgagcctgaaagccaaagcctttgtcatcgtcaaaggcatcgtcgccgtcaaaccgtatagcacggccacgaaagtcggcgtccagccggtcctgccggaaaaagccacgctgctgtatagcgacggcacgacgaaaggcgccacggtcacgtgggacgaaatcccggaagacaaactggccaaagaaggccgctttacggtcgaaggcagcgtcgaaggcacggacctgaaagccaacgtctatgtccgcgtcacgaacgaagtcaaaagcgtcaacatcatgctgcaggaacagggcagcgcctatccgaaactggaagccacgtttacgaacccggccgacaacctgcagcatctgaacgacggcatcaaaagctatacgaacaacccggtcaaccgctggacgaactggacgcgcacgccgcgcgacgccggcgacagcatcacggtcaactttggcaaaaaacatgtcatcaacaacctggacctgtttgtctttacggacagcggcacggtcgtcccggaaaaagccgaagtccagtattgggacggcacggcctggaaagacgtcgaaaacctgacgcagccgagcccgtatgtcgtcgaaaaaaacgaactgacgtttgacgccgtcgccacggaaaaactgaaatttcatctgacgccgagcgtcaaaggcaaatttctggccctgacggaagccgaagtctatgccgaccagatcgtcatgggcgaaacggccaaactgcagagcatcacggtcaacggcaaagccctggaaggctttgaccatgccaaaaaaaactatgaactggtcctgccgtatggcagcgaactgccgaaaatcgaagccgccgccgccgacaacgccacggtcacgatcctgccggcctttagctatccgggcacggccaaactgtttgtcacgagcgaagacggcaaagtcacgacggaatatagcatcggcgtcagcacggaagaaccgaaactggtcagcgccgaactgagcgccgacaaaacgaacgtcatggaagacgacatcatcgacctgaaagtcatcggcctgtttgaaagcaaagaaaaaatcgacgtcacggacagccagccgacgtatgaatttgaccagcagatcatcaaaatcgaaggcaacaaactgtatgccctggaaacgggcaacgtcaaagtcaaagtcacggtcacgtataaaggcgtcagcgtcacgacgccggccctggaatttacgatcgccaaaaacccggccccgaaatatatcacgagcctggaaccggtcacggtcgtcgtcaaaaaaggcgaagccccggaactgccggccacggtcgtcgcccattataaccgcggcatcccgcgcgacgtcaaagtcaaatgggaacgcatcaacccgagcaaatatcagcagctgggcgaatttacggtcagcggcatggtcgaaggcacggacatcaaagcccaggccaaagtcatcgtcaaaggcgccgtcgccgtcgaagacatccgcatggccgtcctgctgaaacagatgccgcagctgccgggcaaagtcacggtctattatagcgacggcgccgaagaacagcgcgccgtcaaatgggaagaaatcccgcaggaagaactggaaaacgtcggcgaatttaaagtcaaaggcgacgtcaacggcgtcaaactgaaagccacggccacgatccgcgtcacggacgaagtcggcggcgaacagaacatcagccgcgccaaaaacggctatgaatatccgaaagccgaagccagctttacgaacaacggcccaggcagcagcgaccgcatcgaagccatcaacgacgacgtcatcagctatgaagccaacccgcataaccgctggacgaactggcagccggtcccgcgcgccggcgactgggtcagcatcacgtttggcgactatgaaccgacggaatatgacgtcgacagcatggaaatccattggtttgccgaccatggcacgagctatccggaacgctttcagatcgaatataaaagcggcgacagctggaaagaagtcacgagcctgaaaagcgacccggccagcccggccctgggcaaagccaacgtctatagctttgaccgcgtcaaaacgagcgccatccgcgtcaaaatgacggcccaggccggcaaaagcctggccatcacggaactgaaagtctttagcaaatggccgaaagccggcacggaaccggaagtcacggacatcaaagtcggcggcaaaagcatcctggaagactttgaacagaaaggcgaccattatgaagtcacgatcgacgccggcgacgccaacgtcatgccgaaaatcaacgtcaaagccaaagaccagacgagcatcacgatcgtcccggccgtcacgagcccgagcacggccaaagtcatcgccaaaagcgaagacggcaaaaaagtcaaagtctatagcatccattataaataa

SEQ ID NO: 8 - protein, 1710 aa, B. circulans ATCC 31382
MSKTTSAAGNSVSYDGERRVNFNENWRFQRETNGSIAGAQNPGFDDSSWRKLNLPHDWSIELDFNKNSLATHEGGYLDGGIGWYRKTFTIPESMKGKRISLDFDGVYMNSTTYLNGEVLGTYPFGYNAFSYDISDKLYKDGRANVLVVKVNNTQPSSRWYSGSGIYRNVYLTVTDPIHVARYGTFVTTPNLEKSIKEDRADVNIKTKISNDAAEAKQVKIKSTIYDGAGNTVQTVETEEKTAAAGTVTPFEQNTVIKQPKLWSIDKPYRYNLVTEVIVGGQTVDTYETKFGVRYFKFDENEGFSLNGEYMKLHGVSMHHDLGALGAATNARGVERQMQIMKDMGVNAIRVTHNPASPELLEAANKLGLFIIEEAFDSWAQSKKPYDYGRFFNAWAEHDIKEMVDRGKNEPAIIMWSIGNEIYDTTNAAGVETARNLVGWVKEIDTTRPTTIGEDKTRGDKVNVTPINSYIKEIFNIVDVVGLNYSENNYDGYHKQNPSWKLYGSETSSATRSRGVYTHPYQYNQSTKYADLQQSSYDNDYVGWGRTAEDAWKYDRDLKHIAGQFIWTGFDYIGEPTPYYNSYPAKSSYFGAVDTAGFPKDIFYYYQSQWKKEPMVHLLPHWNWKEGEKVRVLAYTNASKVELVLNGESLGEKNYDNKQTSWGAPYKETKDGKTYLEWAVPFKPGKLEAVAKDENGKVIARDQVVTAGEPASVRLTADRKVVKADGTDLSFITADIVDSKGIVVPDADHLITFNVTGQGELAGVDNGNASSVERYKDNKRKAFSGKALAIVQSSKLSGKITVHASVAGLSSDSTSVFTVTPADHDKKIVAGIDDVNLTVDVNEAPKLPSEIKVYYSDESAAAKNVTWDEVDPKQYSTVGEFTVEGSVEGTSLKAKAFVIVKGIVAVKPYSTATKVGVQPVLPEKATLLYSDGTTKGATVTWDEIPEDKLAKEGRFTVEGSVEGTDLKANVYVRVTNEVKSVNIMLQEQGSAYPKLEATFTNPADNLQHLNDGIKSYTNNPVNRWTNWTRTPRDAGDSITVNFGKKHVINNLDLFVFTDSGTVVPEKAEVQYWDGTAWKDVENLTQPSPYVVEKNELTFDAVATEKLKFHLTPSVKGKFLALTEAEVYADQIVMGETAKLQSITVNGKALEGFDHAKKNYELVLPYGSELPKIEAAAADNATVTILPAFSYPGTAKLFVTSEDGKVTTEYSIGVSTEEPKLVSAELSADKTNVMEDDIIDLKVIGLFESKEKIDVTDSQPTYEFDQQIIKIEGNKLYALETGNVKVKVTVTYKGVSVTTPALEFTIAKNPAPKYITSLEPVTVVVKKGEAPELPATVVAHYNRGIPRDVKVKWERINPSKYQQLGEFTVSGMVEGTDIKAQAKVIVKGAVAVEDIRMAVLLKQMPQLPGKVTVYYSDGAEEQRAVKWEEIPQEELENVGEFKVKGDVNGVKLKATATIRVTDEVGGEQNISRAKNGYEYPKAEASFTNNGPGSSDRIEAINDDVISYEANPHNRWTNWQPVPRAGDWVSITFGDYEPTEYDVDSMEIHWFADHGTSYPERFQIEYKSGDSWKEVTSLKSDPASPALGKANVYSFDRVKTSAIRVKMTAQAGKSLAITELKVFSKWPKAGTEPEVTDIKVGGKSILEDFEQKGDHYEVTIDAGDANVMPKINVKAKDQTSITIVPAVTSPSTAKVIAKSEDGKKVKVYSIHYK

SEQ ID NO: 9 - DNA, 3669 bp, Artificial Sequence
  The sequence is synthesized
atgagcaaaacgacgagcgccgccggcaacagcgtcagctatgacggcgaacgccgcgtcaactttaacgaaaactggcgctttcagcgcgaaacgaacggcagcatcgccggcgcccagaacccaggctttgacgacagcagctggcgcaaactgaacctgccgcatgactggagcatcgaactggactttaacaaaaacagcctggccacgcatgaaggcggctatctggacggcggcatcggctggtatcgcaaaacgtttacgatcccggaaagcatgaaaggcaaacgcatcagcctggactttgacggcgtctatatgaacagcacgacgtatctgaacggcgaagtcctgggcacgtatccgtttggctataacgcctttagctatgacatcagcgacaaactgtataaagacggccgcgccaacgtcctggtcgtcaaagtcaacaacacgcagccgagcagccgctggtatagcggcagcggcatctatcgcaacgtctatctgacggtcacggacccgatccatgtcgcccgctatggcacgtttgtcacgacgccgaacctggaaaaaagcatcaaagaagaccgcgccgacgtcaacatcaaaacgaaaatcagcaacgacgccgccgaagccaaacaggtcaaaatcaaaagcacgatctatgacggcgccggcaacacggtccagacggtcgaaacggaagaaaaaacggccgccgccggcacggtcacgccgtttgaacagaacacggtcatcaaacagccgaaactgtggagcatcgacaaaccgtatcgctataacctggtcacggaagtcatcgtcggcggccagacggtcgacacgtatgaaacgaaatttggcgtccgctattttaaatttgacgaaaacgaaggctttagcctgaacggcgaatatatgaaactgcatggcgtcagcatgcatcatgacctgggcgccctgggcgccgccacgaacgcccgcggcgtcgaacgccagatgcagatcatgaaagacatgggcgtcaacgccatccgcgtcacgcataacccggccagcccggaactgctggaagccgccaacaaactgggcctgtttatcatcgaagaagcctttgacagctgggcccagagcaaaaaaccgtatgactatggccgcttttttaacgcctgggccgaacatgacatcaaagaaatggtcgaccgcggcaaaaacgaaccggccatcatcatgtggagcatcggcaacgaaatctatgacacgacgaacgccgccggcgtcgaaacggcccgcaacctggtcggctgggtcaaagaaatcgacacgacgcgcccgacgacgatcggcgaagacaaaacgcgcggcgacaaagtcaacgtcacgccgatcaacagctatatcaaagaaatctttaacatcgtcgacgtcgtcggcctgaactatagcgaaaacaactatgacggctatcataaacagaacccgagctggaaactgtatggcagcgaaacgagcagcgccacgcgcagccgcggcgtctatacgcatccgtatcagtataaccagagcacgaaatatgccgacctgcagcagagcagctatgacaacgactatgtcggctggggccgcacggccgaagacgcctggaaatatgaccgcgacctgaaacatatcgccggccagtttatctggacgggctttgactatatcggcgaaccgacgccgtattataacagctatccggccaaaagcagctattttggcgccgtcgacacggccggctttccgaaagacatcttttattattatcagagccagtggaaaaaagaaccgatggtccatctgctgccgcattggaactggaaagaaggcgaaaaagtccgcgtcctggcctatacgaacgccagcaaagtcgaactggtcctgaacggcgaaagcctgggcgaaaaaaactatgacaacaaacagacgagctggggcgccccgtataaagaaacgaaagacggcaaaacgtatctggaatgggccgtcccgtttaaaccgggcaaactggaagccgtcgccaaagacgaaaacggcaaagtcatcgcccgcgaccaggtcgtcacggccggcgaaccggccagcgtccgcctgacggccgaccgcaaagtcgtcaaagccgacggcacggacctgagctttatcacggccgacatcgtcgacagcaaaggcatcgtcgtcccggacgccgaccatctgatcacgtttaacgtcacgggccagggcgaactggccggcgtcgacaacggcaacgccagcagcgtcgaacgctataaagacaacaaacgcaaagcctttagcggcaaagccctggccatcgtccagagcagcaaactgagcggcaaaatcacggtccatgccagcgtcgccggcctgagcagcgacagcacgagcgtctttacggtcacgccggccgaccatgacaaaaaaatcgtcgccggcatcgacgacgtcaacctgacggtcgacgtcaacgaagccccgaaactgccgagcgaaatcaaagtctattatagcgacgaaagcgccgccgccaaaaacgtcacgtgggacgaagtcgacccgaaacagtatagcacggtcggcgaatttacggtcgaaggcagcgtcgaaggcacgagcctgaaagccaaagcctttgtcatcgtcaaaggcatcgtcgccgtcaaaccgtatagcacggccacgaaagtcggcgtccagccggtcctgccggaaaaagccacgctgctgtatagcgacggcacgacgaaaggcgccacggtcacgtgggacgaaatcccggaagacaaactggccaaagaaggccgctttacggtcgaaggcagcgtcgaaggcacggacctgaaagccaacgtctatgtccgcgtcacgaacgaagtcaaaagcgtcaacatcatgctgcaggaacagggcagcgcctatccgaaactggaagccacgtttacgaacccggccgacaacctgcagcatctgaacgacggcatcaaaagctatacgaacaacccggtcaaccgctggacgaactggacgcgcacgccgcgcgacgccggcgacagcatcacggtcaactttggcaaaaaacatgtcatcaacaacctggacctgtttgtctttacggacagcggcacggtcgtcccggaaaaagccgaagtccagtattgggacggcacggcctggaaagacgtcgaaaacctgacgcagccgagcccgtatgtcgtcgaaaaaaacgaactgacgtttgacgccgtcgccacggaaaaactgaaatttcatctgacgccgagcgtcaaaggcaaatttctggccctgacggaagccgaagtctatgccgaccagatcgtcatgggcgaaacggccaaactgcagagcatcacggtcaacggcaaagccctggaaggctttgaccatgccaaaaaaaactatgaactggtcctgccgtatggcagcgaactgccgaaaatcgaagccgccgccgccgacaacgccacggtcacgatcctgccggcctttagctatccgggcacggccaaactgtttgtcacgagcgaagacggcaaagtcacgacggaatatagcatcggcgtcagcacggaagaaccgaaactggtcagcgcctaa

SEQ ID NO: 10 - protein, 1222 aa, Artificial Sequence
  The sequence is synthesized
MSKTTSAAGNSVSYDGERRVNFNENWRFQRETNGSIAGAQNPGFDDSSWRKLNLPHDWSIELDFNKNSLATHEGGYLDGGIGWYRKTFTIPESMKGKRISLDFDGVYMNSTTYLNGEVLGTYPFGYNAFSYDISDKLYKDGRANVLVVKVNNTQPSSRWYSGSGIYRNVYLTVTDPIHVARYGTFVTTPNLEKSIKEDRADVNIKTKISNDAAEAKQVKIKSTIYDGAGNTVQTVETEEKTAAAGTVTPFEQNTVIKQPKLWSIDKPYRYNLVTEVIVGGQTVDTYETKFGVRYFKFDENEGFSLNGEYMKLHGVSMHHDLGALGAATNARGVERQMQIMKDMGVNAIRVTHNPASPELLEAANKLGLFIIEEAFDSWAQSKKPYDYGRFFNAWAEHDIKEMVDRGKNEPAIIMWSIGNEIYDTTNAAGVETARNLVGWVKEIDTTRPTTIGEDKTRGDKVNVTPINSYIKEIFNIVDVVGLNYSENNYDGYHKQNPSWKLYGSETSSATRSRGVYTHPYQYNQSTKYADLQQSSYDNDYVGWGRTAEDAWKYDRDLKHIAGQFIWTGFDYIGEPTPYYNSYPAKSSYFGAVDTAGFPKDIFYYYQSQWKKEPMVHLLPHWNWKEGEKVRVLAYTNASKVELVLNGESLGEKNYDNKQTSWGAPYKETKDGKTYLEWAVPFKPGKLEAVAKDENGKVIARDQVVTAGEPASVRLTADRKVVKADGTDLSFITADIVDSKGIVVPDADHLITFNVTGQGELAGVDNGNASSVERYKDNKRKAFSGKALAIVQSSKLSGKITVHASVAGLSSDSTSVFTVTPADHDKKIVAGIDDVNLTVDVNEAPKLPSEIKVYYSDESAAAKNVTWDEVDPKQYSTVGEFTVEGSVEGTSLKAKAFVIVKGIVAVKPYSTATKVGVQPVLPEKATLLYSDGTTKGATVTWDEIPEDKLAKEGRFTVEGSVEGTDLKANVYVRVTNEVKSVNIMLQEQGSAYPKLEATFTNPADNLQHLNDGIKSYTNNPVNRWTNWTRTPRDAGDSITVNFGKKHVINNLDLFVFTDSGTVVPEKAEVQYWDGTAWKDVENLTQPSPYVVEKNELTFDAVATEKLKFHLTPSVKGKFLALTEAEVYADQIVMGETAKLQSITVNGKALEGFDHAKKNYELVLPYGSELPKIEAAAADNATVTILPAFSYPGTAKLFVTSEDGKVTTEYSIGVSTEEPKLVSA

SEQ ID NO: 11 - DNA, 2463 bp, Artificial Sequence
  The sequence is synthesized
atgagcaaaacgacgagcgccgccggcaacagcgtcagctatgacggcgaacgccgcgtcaactttaacgaaaactggcgctttcagcgcgaaacgaacggcagcatcgccggcgcccagaacccaggctttgacgacagcagctggcgcaaactgaacctgccgcatgactggagcatcgaactggactttaacaaaaacagcctggccacgcatgaaggcggctatctggacggcggcatcggctggtatcgcaaaacgtttacgatcccggaaagcatgaaaggcaaacgcatcagcctggactttgacggcgtctatatgaacagcacgacgtatctgaacggcgaagtcctgggcacgtatccgtttggctataacgcctttagctatgacatcagcgacaaactgtataaagacggccgcgccaacgtcctggtcgtcaaagtcaacaacacgcagccgagcagccgctggtatagcggcagcggcatctatcgcaacgtctatctgacggtcacggacccgatccatgtcgcccgctatggcacgtttgtcacgacgccgaacctggaaaaaagcatcaaagaagaccgcgccgacgtcaacatcaaaacgaaaatcagcaacgacgccgccgaagccaaacaggtcaaaatcaaaagcacgatctatgacggcgccggcaacacggtccagacggtcgaaacggaagaaaaaacggccgccgccggcacggtcacgccgtttgaacagaacacggtcatcaaacagccgaaactgtggagcatcgacaaaccgtatcgctataacctggtcacggaagtcatcgtcggcggccagacggtcgacacgtatgaaacgaaatttggcgtccgctattttaaatttgacgaaaacgaaggctttagcctgaacggcgaatatatgaaactgcatggcgtcagcatgcatcatgacctgggcgccctgggcgccgccacgaacgcccgcggcgtcgaacgccagatgcagatcatgaaagacatgggcgtcaacgccatccgcgtcacgcataacccggccagcccggaactgctggaagccgccaacaaactgggcctgtttatcatcgaagaagcctttgacagctgggcccagagcaaaaaaccgtatgactatggccgcttttttaacgcctgggccgaacatgacatcaaagaaatggtcgaccgcggcaaaaacgaaccggccatcatcatgtggagcatcggcaacgaaatctatgacacgacgaacgccgccggcgtcgaaacggcccgcaacctggtcggctgggtcaaagaaatcgacacgacgcgcccgacgacgatcggcgaagacaaaacgcgcggcgacaaagtcaacgtcacgccgatcaacagctatatcaaagaaatctttaacatcgtcgacgtcgtcggcctgaactatagcgaaaacaactatgacggctatcataaacagaacccgagctggaaactgtatggcagcgaaacgagcagcgccacgcgcagccgcggcgtctatacgcatccgtatcagtataaccagagcacgaaatatgccgacctgcagcagagcagctatgacaacgactatgtcggctggggccgcacggccgaagacgcctggaaatatgaccgcgacctgaaacatatcgccggccagtttatctggacgggctttgactatatcggcgaaccgacgccgtattataacagctatccggccaaaagcagctattttggcgccgtcgacacggccggctttccgaaagacatcttttattattatcagagccagtggaaaaaagaaccgatggtccatctgctgccgcattggaactggaaagaaggcgaaaaagtccgcgtcctggcctatacgaacgccagcaaagtcgaactggtcctgaacggcgaaagcctgggcgaaaaaaactatgacaacaaacagacgagctggggcgccccgtataaagaaacgaaagacggcaaaacgtatctggaatgggccgtcccgtttaaaccgggcaaactggaagccgtcgccaaagacgaaaacggcaaagtcatcgcccgcgaccaggtcgtcacggccggcgaaccggccagcgtccgcctgacggccgaccgcaaagtcgtcaaagccgacggcacggacctgagctttatcacggccgacatcgtcgacagcaaaggcatcgtcgtcccggacgccgaccatctgatcacgtttaacgtcacgggccagggcgaactggccggcgtcgacaacggcaacgccagcagcgtcgaacgctataaagacaacaaacgcaaagcctttagcggcaaagccctggccatcgtccagagcagcaaactgagcggcaaaatcacggtccatgccagcgtcgccggcctgagcagcgacagcacgagcgtctttacggtcacgccgtaa

SEQ ID NO: 12 - protein, 820 aa, Artificial Sequence
  The sequence is synthesized
MSKTTSAAGNSVSYDGERRVNFNENWRFQRETNGSIAGAQNPGFDDSSWRKLNLPHDWSIELDFNKNSLATHEGGYLDGGIGWYRKTFTIPESMKGKRISLDFDGVYMNSTTYLNGEVLGTYPFGYNAFSYDISDKLYKDGRANVLVVKVNNTQPSSRWYSGSGIYRNVYLTVTDPIHVARYGTFVTTPNLEKSIKEDRADVNIKTKISNDAAEAKQVKIKSTIYDGAGNTVQTVETEEKTAAAGTVTPFEQNTVIKQPKLWSIDKPYRYNLVTEVIVGGQTVDTYETKFGVRYFKFDENEGFSLNGEYMKLHGVSMHHDLGALGAATNARGVERQMQIMKDMGVNAIRVTHNPASPELLEAANKLGLFIIEEAFDSWAQSKKPYDYGRFFNAWAEHDIKEMVDRGKNEPAIIMWSIGNEIYDTTNAAGVETARNLVGWVKEIDTTRPTTIGEDKTRGDKVNVTPINSYIKEIFNIVDVVGLNYSENNYDGYHKQNPSWKLYGSETSSATRSRGVYTHPYQYNQSTKYADLQQSSYDNDYVGWGRTAEDAWKYDRDLKHIAGQFIWTGFDYIGEPTPYYNSYPAKSSYFGAVDTAGFPKDIFYYYQSQWKKEPMVHLLPHWNWKEGEKVRVLAYTNASKVELVLNGESLGEKNYDNKQTSWGAPYKETKDGKTYLEWAVPFKPGKLEAVAKDENGKVIARDQVVTAGEPASVRLTADRKVVKADGTDLSFITADIVDSKGIVVPDADHLITFNVTGQGELAGVDNGNASSVERYKDNKRKAFSGKALAIVQSSKLSGKITVHASVAGLSSDSTSVFTVTP

SEQ ID NO: 13 - DNA, 5132 bp, Artificial Sequence
  The sequence is synthesized
atgaaaagtacaaccagtgcagccggtaaatccgttagttataacgacggagagcgtagagtgaattttgagaattggcggttccaacgcgagacgaatggcagtattgcaggtgcgcagaacccaggttttgatgattcatcatggagaaaacttaatctgccgcatgaatggtctatcgatttagactttaataaaaacagtttggctacgcatgaaggaggttaccttgatgggggaattggctggaatagaaaaacgtttacaattccggagtcgatgaaagggaagcggttttctttggactttgatggtgtctacatgaactccactacctaccttaacggtgaagttttgggtacttacccattcggatacaacgccttctcttacgacatttccgacaagttgtacaaagatggcagagcaaacgtgttggtcgtcaaagttaacacgaatcagcctagcggacgctggtatagcggatcatcaatttatagaaacgtctatcttacggtgaccgacccgatccatgtggcgagatacggcacgtttgtaacaacaccaaatctggaaaaaagtatcaaggaagaccgggatgcagttaacattaaaacgaagatcagcaacgcagaagccaagcaagtcaaaatcgctattaagtctactatctacgatggtgctggtaacaccgtccaaactgttgaaaccgaggaaaagacagcagctgctggtacagtcactccattcgagcagaacaccgttattaagcaacctaagttgtggtccatcgacaaaccatacagatacaacttggtcactgaagttattgtaggaggtcagacggtcgatacatatgagacgaagtttggagtccggtacttcaaatttgatgaaaacgaaggctattcattgaacggtgaatttatgaaactccacggagtctcgatgcatcacgatttggctggaggtgcggcgcttacaaatgcaagaggcgtcgaaagacaaatgcaaattatgaaggatgttggagtcaacgcgattagagttacgcataaccctgcttcaccagaattaggcttagaatttgcggccaacaaattattaatcattgaggaggcatttgattcttgggcgcagtctaaaaaaccgtatgactatggccgcttttttaatgcttgggctgagcatgatattaaggaaatggtcgatagaggtaaaaacgaacctgcgatcataatgtggagcataggaaacgagatatatgacactactaatgcagctggagttgagactgctcgaaatctcgttggctgggtaaaagaaatcgacacaacgccgagagccacaattggggaagataaaacccgaggagataatgtgacaccgattaactcatatattaaagaaatcttcaacattgtggacgtcgttggtctcaactactccgaaaacaactacgatggataccacaagcagaacccatcttggaagttgtacggttccgagaccagttccgctactagatccagaggtgtctacacccatccttaccaatacaaccatgatacaaaatatgcggatttgcagcagtcttcgtatgacaatgattatgttggatggggtagaacagcacaggatgcttggaaatatgatcgtgatcttaaacatattgcaggtcaatttatttggacaggcttcgattatattggagaaccaacaccgtattataactcatacccggcaaaaagctcatatttcggagcagttgacacggcagggttccctaaagacattttctattattaccaaagccagtggaaaaaagaacctatggttcaccttttgccgcactggaactggaaagagggagagaaggttcgggtattggcgtataccaatgcgagcaaagttgaacttgtgctgaatggagaatcactcggcaacgaaaagtatgataacaagcaaactagttggggtgcgccgtacaaagaaacaaaagatggtaaaacatacttagaatgggcagtcccattcaagcctggaaagttggaagctgttgccaaggatgagaatggtaaggtcattgcaagagatcaagttgtcaccgctggtgaaccagcctccgttagattgactgctgacagaaaggtcgttaaggctgatggtactgacttgtcgttcatcactgctgacattgtcgactccaaaggcatcgtcgtcccggacgcagatcatctgattacgtttaacgtgacaggacagggtgaacttgcgggggttgataatggtaatgcgtcttcagttgaacgctacaaagataataaaagaaaggcattttcggggaaagcgttggccatcgtgcagagctcaaaactgagcggcaagataaccgtacatgcatctgtggctggcttaagctccgatagcacatccgtgttcactgtaacccctgccgatcacgataagaaaatcgtggccggaattgatgacgtgaatctgacggttgatgtcaatgaagcccctaagcttccgagcgagattaaggtctattactccgatgaatcagccgcggctaaaaacgttacatgggatgaagttgatcctaagcaatatagcaccgtcggcgagtttacagtcgaagggtctgtcgaaggtacaagcttaaaagctaaagcattcgtaattgttaagggaattgtcgctgtcaagccgtactcgactgccacaaaggtaggagtccagccggtcttacctgaaaaagcgaccctgctttattcagacggcacaaccaaaggcgcgacagtgacatgggacgagctgcctgaggataagcttgctaaagagggtcggttcaccgtggaaggctcggtagaaggcaccgatttaaaagcaaatgtctacgttcgcgtgactaacgaagttaaatcagtcaatattatgcttcaagaacaaggatcagcttatccaaagttagaggctacatttacgaatcctgcggataaccttcaacatctgaacgacggcattaagagttatacgaataaccaggtgaaccgctggacaaattggactagaaccccaagagacgctggtgacagcatcacagtgaattttggcaagaagcacgtcattaacaacttggacttgttcgttttcaccgactctggtactgtcgttcctgagaaggctgaagtccagtactgggatggtactgcctggaaagacgttgagaacttgactcaaccatccccatacgtcgttgaaaagaacgagttgaccttcgatgctgtcgctactgaaaagttgaagttccacttgacaccttctgttaagggaaagttcctcgccctgaccgaagccgaggtgtatgcggaccagatcgttgatggggaaacagcgaaacttcaatctattaccgtgaacggcaaagccttggagggttttgatcatgcaaagaaaaactatgaattggtcctcccgtacggatcggagctcccgaagatagaagcagcggctgccgataatgcgaccgtgacaattttgccagcattcagctatccgggcacggctaaattatttgtcacgagtgaagatggaaaggtgaccactgaatattctatcggggtatctactgaagaaccaaaattagtgagcgcggaattaagtgcggataaaacgaacgttatggaagacgatattattgatcttaaggtgattggtctttttgaatctaaggaaaaaattgatgtgacagactcacaaccaacatacgaatttgatcagcagattattaagattgaaggaaacaaactgtatgctttggagaccggcaatgtgaaagtcaaggttacagttacatataaaggcgtctcagttacaacgccggctcttgagtttacaatagctaaacaccctgcgccaaaatatatcacatcactggaacctgttacggtggttgttaaaaaaggtgaggcgccagaactgcctgctactgtcgtagcgcactataatcggggcattccgcgcgacgtaaaagtgaaatgggagcgtattcatccttcaaaatatcaacaactgggggagttcacagtatcaggaatggtcgaaggtactgacattaaagctcaagccaaagtagcggtcaaaggagcggtcatcgtagaagatattagaatggcagttcttttgaaacagatgccacaattaccgggaaaagttactgtctattactctgacggagccgaggagcaacgggccgttaaatgggaagaaattccacaggaagagctggagaaagtaggagagttcaaagtcaatggtgatgttaatggcgttaaattaaaggccactgctacaatacgggtgactgacgaggtcggagctgaacaaaacataagccgggcgaaaaacggctatgaatacccgaaagccgaagcatcctttacgaatgatggtccgggctcctccgatagaatcgaggccattaacgacgacgtcatctcttacgaagccaacccacacaacagatggaccaactggcaacctgttccaagagctggtgactgggtatccattaccttcggtgactacgagccaaccgaatacgacgttgactctatggagatccactggttcgctgaccacggtacttcctaccctgaacgttttcaaattgaatataaatcaggagactcctggaaagaagtaacaagcctgaaaagtgacccagcttccccagctttagggaaagctaatgtgtactcgtttgatcgcgttaagacgtcagccattcgggtaaaaatgacagcgcaggcaggtaaaagtctggccattaccgaacttaaagtttttagcaaatggccgaaagccggaacagaacctgatgttacagatattaaagtgggtggaaaatccatactggaagagttcgaacaagaaggagaccattatgaagcaacgatagatgtgggcgacgcgaacgtgatgcctaaaatttatgttaaggcgaaagaccaaacaagcatctcaatcgttccggctgtaacgagcgtcagcaccgctaaggtgatcgcagaggacggagacggtaaaaaagtgaaggtttattcgatccataagagctacaataa

SEQ ID NO: 14 - protein, 1709 aa, Artificial Sequence
  The sequence is synthesized
MKSTTSAAGKSVSYNDGERRVNFENWRFQRETNGSIAGAQNPGFDDSSWRKLNLPHEWSIDLDFNKNSLATHEGGYLDGGIGWNRKTFTIPESMKGKRFSLDFDGVYMNSTTYLNGEVLGTYPFGYNAFSYDISDKLYKDGRANVLVVKVNTNQPSGRWYSGSSIYRNVYLTVTDPIHVARYGTFVTTPNLEKSIKEDRDAVNIKTKISNAEAKQVKIAIKSTIYDGAGNTVQTVETEEKTAAAGTVTPFEQNTVIKQPKLWSIDKPYRYNLVTEVIVGGQTVDTYETKFGVRYFKFDENEGYSLNGEFMKLHGVSMHHDLAGGAALTNARGVERQMQIMKDVGVNAIRVTHNPASPELGLEFAANKLLIIEEAFDSWAQSKKPYDYGRFFNAWAEHDIKEMVDRGKNEPAIIMWSIGNEIYDTTNAAGVETARNLVGWVKEIDTTPRATIGEDKTRGDNVTPINSYIKEIFNIVDVVGLNYSENNYDGYHKQNPSWKLYGSETSSATRSRGVYTHPYQYNHDTKYADLQQSSYDNDYVGWGRTAQDAWKYDRDLKHIAGQFIWTGFDYIGEPTPYYNSYPAKSSYFGAVDTAGFPKDIFYYYQSQWKKEPMVHLLPHWNWKEGEKVRVLAYTNASKVELVLNGESLGNEKYDNKQTSWGAPYKETKDGKTYLEWAVPFKPGKLEAVAKDENGKVIARDQVVTAGEPASVRLTADRKVVKADGTDLSFITADIVDSKGIVVPDADHLITFNVTGQGELAGVDNGNASSVERYKDNKRKAFSGKALAIVQSSKLSGKITVHASVAGLSSDSTSVFTVTPADHDKKIVAGIDDVNLTVDVNEAPKLPSEIKVYYSDESAAAKNVTWDEVDPKQYSTVGEFTVEGSVEGTSLKAKAFVIVKGIVAVKPYSTATKVGVQPVLPEKATLLYSDGTTKGATVTWDELPEDKLAKEGRFTVEGSVEGTDLKANVYVRVTNEVKSVNIMLQEQGSAYPKLEATFTNPADNLQHLNDGIKSYTNNQVNRWTNWTRTPRDAGDSITVNFGKKHVINNLDLFVFTDSGTVVPEKAEVQYWDGTAWKDVENLTQPSPYVVEKNELTFDAVATEKLKFHLTPSVKGKFLALTEAEVYADQIVDGETAKLQSITVNGKALEGFDHAKKNYELVLPYGSELPKIEAAAADNATVTILPAFSYPGTAKLFVTSEDGKVTTEYSIGVSTEEPKLVSAELSADKTNVMEDDIIDLKVIGLFESKEKIDVTDSQPTYEFDQQIIKIEGNKLYALETGNVKVKVTVTYKGVSVTTPALEFTIAKHPAPKYITSLEPVTVVVKKGEAPELPATVVAHYNRGIPRDVKVKWERIHPSKYQQLGEFTVSGMVEGTDIKAQAKVAVKGAVIVEDIRMAVLLKQMPQLPGKVTVYYSDGAEEQRAVKWEEIPQEELEKVGEFKVNGDVNGVKLKATATIRVTDEVGAEQNISRAKNGYEYPKAEASFTNDGPGSSDRIEAINDDVISYEANPHNRWTNWQPVPRAGDWVSITFGDYEPTEYDVDSMEIHWFADHGTSYPERFQIEYKSGDSWKEVTSLKSDPASPALGKANVYSFDRVKTSAIRVKMTAQAGKSLAITELKVFSKWPKAGTEPDVTDIKVGGKSILEEFEQEGDHYEATIDVGDANVMPKIYVKAKDQTSISIVPAVTSVSTAKVIAEDGDGKKVKVYSIHKSY

SEQ ID NO: 15 - DNA, 3669 bp, Artificial Sequence
  The sequence is synthesized
atgaaaagcacgacgagcgccgccggcaaaagcgtcagctataacgacggcgaacgccgcgtcaactttgaaaactggcgctttcagcgcgaaacgaacggcagcatcgccggcgcccagaacccaggctttgacgacagcagctggcgcaaactgaacctgccgcatgaatggagcatcgacctggactttaacaaaaacagcctggccacgcatgaaggcggctatctggacggcggcatcggctggaaccgcaaaacgtttacgatcccggaaagcatgaaaggcaaacgctttagcctggactttgacggcgtctatatgaacagcacgacgtatctgaacggcgaagtcctgggcacgtatccgtttggctataacgcctttagctatgacatcagcgacaaactgtataaagacggccgcgccaacgtcctggtcgtcaaagtcaacacgaaccagccgagcggccgctggtatagcggcagcagcatctatcgcaacgtctatctgacggtcacggacccgatccatgtcgcccgctatggcacgtttgtcacgacgccgaacctggaaaaaagcatcaaagaagaccgcgacgccgtcaacatcaaaacgaaaatcagcaacgccgaagccaaacaggtcaaaatcgccatcaaaagcacgatctatgacggcgccggcaacacggtccagacggtcgaaacggaagaaaaaacggccgccgccggcacggtcacgccgtttgaacagaacacggtcatcaaacagccgaaactgtggagcatcgacaaaccgtatcgctataacctggtcacggaagtcatcgtcggcggccagacggtcgacacgtatgaaacgaaatttggcgtccgctattttaaatttgacgaaaacgaaggctatagcctgaacggcgaatttatgaaactgcatggcgtcagcatgcatcatgacctggccggcggcgccgccctgacgaacgcccgcggcgtcgaacgccagatgcagatcatgaaagacgtcggcgtcaacgccatccgcgtcacgcataacccggccagcccggaactgggcctggaatttgccgccaacaaactgctgatcatcgaagaagcctttgacagctgggcccagagcaaaaaaccgtatgactatggccgcttttttaacgcctgggccgaacatgacatcaaagaaatggtcgaccgcggcaaaaacgaaccggccatcatcatgtggagcatcggcaacgaaatctatgacacgacgaacgccgccggcgtcgaaacggcccgcaacctggtcggctgggtcaaagaaatcgacacgacgccgcgcgccacgatcggcgaagacaaaacgcgcggcgacaacgtcacgccgatcaacagctatatcaaagaaatctttaacatcgtcgacgtcgtcggcctgaactatagcgaaaacaactatgacggctatcataaacagaacccgagctggaaactgtatggcagcgaaacgagcagcgccacgcgcagccgcggcgtctatacgcatccgtatcagtataaccatgacacgaaatatgccgacctgcagcagagcagctatgacaacgactatgtcggctggggccgcacggcccaggacgcctggaaatatgaccgcgacctgaaacatatcgccggccagtttatctggacgggctttgactatatcggcgaaccgacgccgtattataacagctatccggccaaaagcagctattttggcgccgtcgacacggccggctttccgaaagacatcttttattattatcagagccagtggaaaaaagaaccgatggtccatctgctgccgcattggaactggaaagaaggcgaaaaagtccgcgtcctggcctatacgaacgccagcaaagtcgaactggtcctgaacggcgaaagcctgggcaacgaaaaatatgacaacaaacagacgagctggggcgccccgtataaagaaacgaaagacggcaaaacgtatctggaatgggccgtcccgtttaaaccgggcaaactggaagccgtcgccaaagacgaaaacggcaaagtcatcgcccgcgaccaggtcgtcacggccggcgaaccggccagcgtccgcctgacggccgaccgcaaagtcgtcaaagccgacggcacggacctgagctttatcacggccgacatcgtcgacagcaaaggcatcgtcgtcccggacgccgaccatctgatcacgtttaacgtcacgggccagggcgaactggccggcgtcgacaacggcaacgccagcagcgtcgaacgctataaagacaacaaacgcaaagcctttagcggcaaagccctggccatcgtccagagcagcaaactgagcggcaaaatcacggtccatgccagcgtcgccggcctgagcagcgacagcacgagcgtctttacggtcacgccggccgaccatgacaaaaaaatcgtcgccggcatcgacgacgtcaacctgacggtcgacgtcaacgaagccccgaaactgccgagcgaaatcaaagtctattatagcgacgaaagcgccgccgccaaaaacgtcacgtgggacgaagtcgacccgaaacagtatagcacggtcggcgaatttacggtcgaaggcagcgtcgaaggcacgagcctgaaagccaaagcctttgtcatcgtcaaaggcatcgtcgccgtcaaaccgtatagcacggccacgaaagtcggcgtccagccggtcctgccggaaaaagccacgctgctgtatagcgacggcacgacgaaaggcgccacggtcacgtgggacgaactgccggaagacaaactggccaaagaaggccgctttacggtcgaaggcagcgtcgaaggcacggacctgaaagccaacgtctatgtccgcgtcacgaacgaagtcaaaagcgtcaacatcatgctgcaggaacagggcagcgcctatccgaaactggaagccacgtttacgaacccggccgacaacctgcagcatctgaacgacggcatcaaaagctatacgaacaaccaggtcaaccgctggacgaactggacgcgcacgccgcgcgacgccggcgacagcatcacggtcaactttggcaaaaaacatgtcatcaacaacctggacctgtttgtctttacggacagcggcacggtcgtcccggaaaaagccgaagtccagtattgggacggcacggcctggaaagacgtcgaaaacctgacgcagccgagcccgtatgtcgtcgaaaaaaacgaactgacgtttgacgccgtcgccacggaaaaactgaaatttcatctgacgccgagcgtcaaaggcaaatttctggccctgacggaagccgaagtctatgccgaccagatcgtcgacggcgaaacggccaaactgcagagcatcacggtcaacggcaaagccctggaaggctttgaccatgccaaaaaaaactatgaactggtcctgccgtatggcagcgaactgccgaaaatcgaagccgccgccgccgacaacgccacggtcacgatcctgccggcctttagctatccgggcacggccaaactgtttgtcacgagcgaagacggcaaagtcacgacggaatatagcatcggcgtcagcacggaagaaccgaaactggtcagcgccgaactgtaa

SEQ ID NO: 16 - protein, 1222 aa, Artificial Sequence
  The sequence is synthesized
MKSTTSAAGKSVSYNDGERRVNFENWRFQRETNGSIAGAQNPGFDDSSWRKLNLPHEWSIDLDFNKNSLATHEGGYLDGGIGWNRKTFTIPESMKGKRFSLDFDGVYMNSTTYLNGEVLGTYPFGYNAFSYDISDKLYKDGRANVLVVKVNTNQPSGRWYSGSSIYRNVYLTVTDPIHVARYGTFVTTPNLEKSIKEDRDAVNIKTKISNAEAKQVKIAIKSTIYDGAGNTVQTVETEEKTAAAGTVTPFEQNTVIKQPKLWSIDKPYRYNLVTEVIVGGQTVDTYETKFGVRYFKFDENEGYSLNGEFMKLHGVSMHHDLAGGAALTNARGVERQMQIMKDVGVNAIRVTHNPASPELGLEFAANKLLIIEEAFDSWAQSKKPYDYGRFFNAWAEHDIKEMVDRGKNEPAIIMWSIGNEIYDTTNAAGVETARNLVGWVKEIDTTPRATIGEDKTRGDNVTPINSYIKEIFNIVDVVGLNYSENNYDGYHKQNPSWKLYGSETSSATRSRGVYTHPYQYNHDTKYADLQQSSYDNDYVGWGRTAQDAWKYDRDLKHIAGQFIWTGFDYIGEPTPYYNSYPAKSSYFGAVDTAGFPKDIFYYYQSQWKKEPMVHLLPHWNWKEGEKVRVLAYTNASKVELVLNGESLGNEKYDNKQTSWGAPYKETKDGKTYLEWAVPFKPGKLEAVAKDENGKVIARDQVVTAGEPASVRLTADRKVVKADGTDLSFITADIVDSKGIVVPDADHLITFNVTGQGELAGVDNGNASSVERYKDNKRKAFSGKALAIVQSSKLSGKITVHASVAGLSSDSTSVFTVTPADHDKKIVAGIDDVNLTVDVNEAPKLPSEIKVYYSDESAAAKNVTWDEVDPKQYSTVGEFTVEGSVEGTSLKAKAFVIVKGIVAVKPYSTATKVGVQPVLPEKATLLYSDGTTKGATVTWDELPEDKLAKEGRFTVEGSVEGTDLKANVYVRVTNEVKSVNIMLQEQGSAYPKLEATFTNPADNLQHLNDGIKSYTNNQVNRWTNWTRTPRDAGDSITVNFGKKHVINNLDLFVFTDSGTVVPEKAEVQYWDGTAWKDVENLTQPSPYVVEKNELTFDAVATEKLKFHLTPSVKGKFLALTEAEVYADQIVDGETAKLQSITVNGKALEGFDHAKKNYELVLPYGSELPKIEAAAADNATVTILPAFSYPGTAKLFVTSEDGKVTTEYSIGVSTEEPKLVSAEL

SEQ ID NO: 17 - DNA, 2463 bp, Artificial Sequence
  The sequence is synthesized
atgaaaagcacgacgagcgccgccggcaaaagcgtcagctataacgacggcgaacgccgcgtcaactttgaaaactggcgctttcagcgcgaaacgaacggcagcatcgccggcgcccagaacccaggctttgacgacagcagctggcgcaaactgaacctgccgcatgaatggagcatcgacctggactttaacaaaaacagcctggccacgcatgaaggcggctatctggacggcggcatcggctggaaccgcaaaacgtttacgatcccggaaagcatgaaaggcaaacgctttagcctggactttgacggcgtctatatgaacagcacgacgtatctgaacggcgaagtcctgggcacgtatccgtttggctataacgcctttagctatgacatcagcgacaaactgtataaagacggccgcgccaacgtcctggtcgtcaaagtcaacacgaaccagccgagcggccgctggtatagcggcagcagcatctatcgcaacgtctatctgacggtcacggacccgatccatgtcgcccgctatggcacgtttgtcacgacgccgaacctggaaaaaagcatcaaagaagaccgcgacgccgtcaacatcaaaacgaaaatcagcaacgccgaagccaaacaggtcaaaatcgccatcaaaagcacgatctatgacggcgccggcaacacggtccagacggtcgaaacggaagaaaaaacggccgccgccggcacggtcacgccgtttgaacagaacacggtcatcaaacagccgaaactgtggagcatcgacaaaccgtatcgctataacctggtcacggaagtcatcgtcggcggccagacggtcgacacgtatgaaacgaaatttggcgtccgctattttaaatttgacgaaaacgaaggctatagcctgaacggcgaatttatgaaactgcatggcgtcagcatgcatcatgacctggccggcggcgccgccctgacgaacgcccgcggcgtcgaacgccagatgcagatcatgaaagacgtcggcgtcaacgccatccgcgtcacgcataacccggccagcccggaactgggcctggaatttgccgccaacaaactgctgatcatcgaagaagcctttgacagctgggcccagagcaaaaaaccgtatgactatggccgcttttttaacgcctgggccgaacatgacatcaaagaaatggtcgaccgcggcaaaaacgaaccggccatcatcatgtggagcatcggcaacgaaatctatgacacgacgaacgccgccggcgtcgaaacggcccgcaacctggtcggctgggtcaaagaaatcgacacgacgccgcgcgccacgatcggcgaagacaaaacgcgcggcgacaacgtcacgccgatcaacagctatatcaaagaaatctttaacatcgtcgacgtcgtcggcctgaactatagcgaaaacaactatgacggctatcataaacagaacccgagctggaaactgtatggcagcgaaacgagcagcgccacgcgcagccgcggcgtctatacgcatccgtatcagtataaccatgacacgaaatatgccgacctgcagcagagcagctatgacaacgactatgtcggctggggccgcacggcccaggacgcctggaaatatgaccgcgacctgaaacatatcgccggccagtttatctggacgggctttgactatatcggcgaaccgacgccgtattataacagctatccggccaaaagcagctattttggcgccgtcgacacggccggctttccgaaagacatcttttattattatcagagccagtggaaaaaagaaccgatggtccatctgctgccgcattggaactggaaagaaggcgaaaaagtccgcgtcctggcctatacgaacgccagcaaagtcgaactggtcctgaacggcgaaagcctgggcaacgaaaaatatgacaacaaacagacgagctggggcgccccgtataaagaaacgaaagacggcaaaacgtatctggaatgggccgtcccgtttaaaccgggcaaactggaagccgtcgccaaagacgaaaacggcaaagtcatcgcccgcgaccaggtcgtcacggccggcgaaccggccagcgtccgcctgacggccgaccgcaaagtcgtcaaagccgacggcacggacctgagctttatcacggccgacatcgtcgacagcaaaggcatcgtcgtcccggacgccgaccatctgatcacgtttaacgtcacgggccagggcgaactggccggcgtcgacaacggcaacgccagcagcgtcgaacgctataaagacaacaaacgcaaagcctttagcggcaaagccctggccatcgtccagagcagcaaactgagcggcaaaatcacggtccatgccagcgtcgccggcctgagcagcgacagcacgagcgtctttacggtcacgccggccgactaa

SEQ ID NO: 18 - protein, 820 aa, Artificial Sequence
  The sequence is synthesized
MKSTTSAAGKSVSYNDGERRVNFENWRFQRETNGSIAGAQNPGFDDSSWRKLNLPHEWSIDLDFNKNSLATHEGGYLDGGIGWNRKTFTIPESMKGKRFSLDFDGVYMNSTTYLNGEVLGTYPFGYNAFSYDISDKLYKDGRANVLVVKVNTNQPSGRWYSGSSIYRNVYLTVTDPIHVARYGTFVTTPNLEKSIKEDRDAVNIKTKISNAEAKQVKIAIKSTIYDGAGNTVQTVETEEKTAAAGTVTPFEQNTVIKQPKLWSIDKPYRYNLVTEVIVGGQTVDTYETKFGVRYFKFDENEGYSLNGEFMKLHGVSMHHDLAGGAALTNARGVERQMQIMKDVGVNAIRVTHNPASPELGLEFAANKLLIIEEAFDSWAQSKKPYDYGRFFNAWAEHDIKEMVDRGKNEPAIIMWSIGNEIYDTTNAAGVETARNLVGWVKEIDTTPRATIGEDKTRGDNVTPINSYIKEIFNIVDVVGLNYSENNYDGYHKQNPSWKLYGSETSSATRSRGVYTHPYQYNHDTKYADLQQSSYDNDYVGWGRTAQDAWKYDRDLKHIAGQFIWTGFDYIGEPTPYYNSYPAKSSYFGAVDTAGFPKDIFYYYQSQWKKEPMVHLLPHWNWKEGEKVRVLAYTNASKVELVLNGESLGNEKYDNKQTSWGAPYKETKDGKTYLEWAVPFKPGKLEAVAKDENGKVIARDQVVTAGEPASVRLTADRKVVKADGTDLSFITADIVDSKGIVVPDADHLITFNVTGQGELAGVDNGNASSVERYKDNKRKAFSGKALAIVQSSKLSGKITVHASVAGLSSDSTSVFTVTPAD

SEQ ID NO: 19 - DNA, 628 bp, Bacillus thuringiensis
gaaacgtaagatgaaaccttagataaaagtgctttttttgttgcaattgaagaattattaatgttaagcttaattaaagataatatctttgaattgtaacgcccctcaaaagtaagaactacaaaaaaagaatacgttatatagaaatatgtttgaaccttcttcagattacaaatatattcggacggactctacctcaaatgcttatctaactatagaatgacatacaagcacaaccttgaaaatttgaaaatataactaccaatgaacttgttcatgtgaattatcgctgtatttaattttctcaattcaatatataatatgccaatacattgttacaagtagaaattaagacacccttgatagccttactatacctaacatgatgtagtattaaatgaatatgtaaatatatttatgataagaagcgacttatttataatcattacatatttttctattggaatgattaagattccaatagaatagtgtataaattatttatcttgaaaggagggatgcctaaaaacgaagaacattaaaaacatatatttgcaccgtctaatggatttatgaaaaatcattttatcagtttgaaaattatgtattatgataagaaagggaggaa

SEQ ID NO: 20 - DNA, 180 bp, Bacillus licheniformis
tttttttataggaacattgatttgtattcactctgccaagttgttttgatagagtgattgtgataattttaaatgtaagcgttaacaaaattctccagtcttcacatcggtttgaaaggaggaagcggaagaatgaagtaagagggatttttgactccgaagtaagtcttcaaaaaatca

SEQ ID NO: 21 - DNA, 426 bp, Bacillus subtilis
tgtcgacgtgcatgcaggccggggcatatgggaaacagcgcggacggagcggaatttccaatttcatgccgcagccgcctgcgctgttctcatttgcggcttccttgtagagctcagcattattgagtggatgattatattccttttgataggtggtatgttttcgcttgaacttttaaatacagccattgaacatacggttgatttaataactgacaaacatcaccctcttgctaaagcggccaaggacgctgccgccggggctgtttgcgtttttaccgtgatttcgtgtatcattggtttacttatttttttgccaaagctgtaatggctgaaaattcttacatttattttacatttttagaaatgggcgtgaaaaaaagcgcgcgattatgtaaaatataaagtgatagcggtaccattata

SEQ ID NO: 22 - DNA, 87 bp, Bacillus licheniformis
atgaaacaacaaaaacggctttacgcccgattgctgccgctgttatttgcgctcatcttcttgctgcctcattctgcagcagcggcg

SEQ ID NO: 23 - DNA, 87 bp, Bacillus licheniformis
atgatgaggaaaaagagtttttggcttgggatgctgacggccttaatgctcgtgttcacgatggccttcagcgattccgcgtctgct

SEQ ID NO: 24 - DNA, 93 bp, Bacillus amyloliquefaciens
atgattcaaaaacgaaagcggacagtttcgttcagacttgtgcttatgtgcacgctgttatttgtcagtttgccgattacaaaaacatcagcc

SEQ ID NO: 25 - DNA, 99 bp, Bacillus subtilis
atgtttgcaaaacgattcaaaacctctttactgccgttattcgctggatttttattgctgtttcatttggttctggcaggaccggcggctgcgagtgct

SEQ ID NO: 26 - DNA, 81 bp, Bacillus licheniformis
gtgggtttaggtaagaaattgtctgttgctgtcgctgcttcgtttatgagtttatcaatcagcctgccaggtgttcaggct

SEQ ID NO: 27 - DNA, 97 bp, Bacillus licheniformis
atgttgatcaacaaaagcaaaaagtttttcgttttttctttcatttttgttatgatgctgagcctctcatttgtgaatggggaagttgcaaaagccg

SEQ ID NO: 28 - DNA, 33 bp, Artificial Sequence
  The sequence is synthesized
ggatcccgggactagttctagagcggccgccac

SEQ ID NO: 29 - DNA, 25 bp, Artificial Sequence
  The sequence is synthesized
gttaagggatgcataaactgcatcc

SEQ ID NO: 30 - DNA, 26 bp, Artificial Sequence
  The sequence is synthesized
gctctagatcaaggcaccgaacgatt

SEQ ID NO: 31 - DNA, 40 bp, Artificial Sequence
  The sequence is synthesized
ctttcgtcttctccatttacgcgctgcacagtttgtattt

SEQ ID NO: 32 - DNA, 42 bp, Artificial Sequence
  The sequence is synthesized
aaatacaaactgtgcagcgcgtaaatggagaagacgcgaaag

SEQ ID NO: 33 - DNA, 26 bp, Artificial Sequence
  The sequence is synthesized
cgggatcctatgcctggtgcctgacg

SEQ ID NO: 34 - DNA, 26 bp, Artificial Sequence
  The sequence is synthesized
gctctagatcaaggcaccgaacgatt

SEQ ID NO: 35 - DNA, 26 bp, Artificial Sequence
  The sequence is synthesized
cgggatcctatgcctggtgcctgacg

SEQ ID NO: 36 - DNA, 24 bp, Artificial Sequence
  The sequence is synthesized
ctgcagattattatgccgctatcc

SEQ ID NO: 37 - DNA, 50 bp, Artificial Sequence
  The sequence is synthesized
tcatcctgtctgacttgaacggcccgggaaatgtattcgtatgggcaagc

SEQ ID NO: 38 - DNA, 50 bp, Artificial Sequence
  The sequence is synthesized
gcttgcccatacgaatacatttcccgggccgttcaagtcagacaggatga

SEQ ID NO: 39 - DNA, 30 bp, Artificial Sequence
  The sequence is synthesized
acgtctagatcttccaaagcgatgatgctc

SEQ ID NO: 40 - DNA, 23 bp, Artificial Sequence
  The sequence is synthesized
cagatgcttggaatgatgaacag

SEQ ID NO: 41 - DNA, 21 bp, Artificial Sequence
  The sequence is synthesized
gacataattgacgcctgcttc

SEQ ID NO: 42 - DNA, 29 bp, Artificial Sequence
  The sequence is synthesized
atttctagaagttcccgtgtaaagagttg

SEQ ID NO: 43 - DNA, 44 bp, Artificial Sequence
  The sequence is synthesized
gcgttacaatggatgaagcccgggtggtttgtatccgctgaatc

SEQ ID NO: 44 - DNA, 44 bp, Artificial Sequence
  The sequence is synthesized
gattcagcggatacaaaccacccgggcttcatccattgtaacgc

SEQ ID NO: 45 - DNA, 28 bp, Artificial Sequence
  The sequence is synthesized
agaggatccagattgatagcctttgccc

SEQ ID NO: 46 - DNA, 20 bp, Artificial Sequence
  The sequence is synthesized
cacccacttcccattatgag

SEQ ID NO: 47 - DNA, 18 bp, Artificial Sequence
  The sequence is synthesized
aaagcggtaaacagccag

SEQ ID NO: 48 - DNA, 31 bp, Artificial Sequence
  The sequence is synthesized
atttctagacggctttatcctttgctgttac

SEQ ID NO: 49 - DNA, 46 bp, Artificial Sequence
  The sequence is synthesized
gaataacgaaaccacaattgacccgggcggaaacctcgctcagaac

SEQ ID NO: 50 - DNA, 45 bp, Artificial Sequence
  The sequence is synthesized
gttctgagcgaggtttccgcccgggtcaatgtggtttcgttattc

SEQ ID NO: 51 - DNA, 29 bp, Artificial Sequence
  The sequence is synthesized
agaggatccagaagagcaaatcaagcaac

SEQ ID NO: 52 - DNA, 18 bp, Artificial Sequence
  The sequence is synthesized
atcatcggaatggttgcg

SEQ ID NO: 53 - DNA, 22 bp, Artificial Sequence
  The sequence is synthesized
actttatcggattgcggagatg

SEQ ID NO: 54 - DNA, 27 bp, Artificial Sequence
  The sequence is synthesized
gctctagaataatccgtgtgttcgccg

SEQ ID NO: 55 - DNA, 39 bp, Artificial Sequence
  The sequence is synthesized
tgatgatgctgactctgcccgggaaaccgttgagatgga

SEQ ID NO: 56 - DNA, 39 bp, Artificial Sequence
  The sequence is synthesized
tccatctcaacggtttcccgggcagagtcagcatcatca

SEQ ID NO: 57 - DNA, 20 bp, Artificial Sequence
  The sequence is synthesized
ttcccagaccacgagttcct

SEQ ID NO: 58 - DNA, 21 bp, Artificial Sequence
  The sequence is synthesized
actggtcaaaggctaaatcgc

SEQ ID NO: 59 - DNA, 19 bp, Artificial Sequence
  The sequence is synthesized
atccatccgcaagtcttcg

SEQ ID NO: 60 - DNA, 28 bp, Artificial Sequence
  The sequence is synthesized
atttctagagattgatttccgccatctc

SEQ ID NO: 61 - DNA, 44 bp, Artificial Sequence
  The sequence is synthesized
tcccgcactcttcaatgagcccgggtcttccttcttcaggctcg

SEQ ID NO: 62 - DNA, 44 bp, Artificial Sequence
  The sequence is synthesized
cgagcctgaagaaggaagacccgggctcattgaagagtgcggga

SEQ ID NO: 63 - DNA, 19 bp, Artificial Sequence
  The sequence is synthesized
aacgagccaaataacgacg

SEQ ID NO: 64 - DNA, 21 bp, Artificial Sequence
  The sequence is synthesized
cgtcaatgaaaaagggctgtc

SEQ ID NO: 65 - DNA, 20 bp, Artificial Sequence
  The sequence is synthesized
acggcgaaaatacggaaaat

SEQ ID NO: 66 - DNA, 28 bp, Artificial Sequence
  The sequence is synthesized
atttctagagccgcttctcatcacacct

SEQ ID NO: 67 - DNA, 41 bp, Artificial Sequence
  The sequence is synthesized
tatggtgctctgttcttccgcattcacatgcattctttccg

SEQ ID NO: 68 - DNA, 41 bp, Artificial Sequence
  The sequence is synthesized
cggaaagaatgcatgtgaatgcggaagaacagagcaccata

SEQ ID NO: 69 - DNA, 21 bp, Artificial Sequence
  The sequence is synthesized
cggcgattcatttattctctg

SEQ ID NO: 70 - DNA, 23 bp, Artificial Sequence
  The sequence is synthesized
atgacaatcagcatctatttggc

SEQ ID NO: 71 - DNA, 20 bp, Artificial Sequence
  The sequence is synthesized
cctcctttctgttcaaccga